European Patent Application EP 4 455 282 A1, published October 30, 2024. Title: 相同組換えを利用したゲノム編集細胞の製造方法. Applicant: OSAKA UNIVERSITY. Application JP. The sequence listing filed with the application follows.

SEQUENCE LISTING (12 sequences)

SEQ ID NO: 1 - DNA, 23 bp, synthetic construct
  misc_feature 1..23: note = Target sequence of sgRNA
  source 1..23: mol_type = other DNA
cgtctcggagcaggcaggcgggg

SEQ ID NO: 2 - DNA, 23 bp, synthetic construct
  misc_feature 1..23: note = Target sequence of sgRNA
  source 1..23: mol_type = other DNA
tcccaccgaaggccacacgccgg

SEQ ID NO: 3 - DNA, 23 bp, synthetic construct
  misc_feature 1..23: note = Target sequence of sgRNA
  source 1..23: mol_type = other DNA
tcaatcatatcactcttagctgg

SEQ ID NO: 4 - DNA, 23 bp, synthetic construct
  misc_feature 1..23: note = Target sequence of sgRNA
  source 1..23: mol_type = other DNA
ggagctgtccatgagacccaggg

SEQ ID NO: 5 - DNA, 23 bp, synthetic construct
  misc_feature 1..23: note = Target sequence of sgRNA
  source 1..23: mol_type = other DNA
ctcgcagaactccagggaactgg

SEQ ID NO: 6 - DNA, 23 bp, synthetic construct
  misc_feature 1..23: note = Target sequence of sgRNA
  source 1..23: mol_type = other DNA
actccacgatgtcagggaactgg

SEQ ID NO: 7 - DNA, 23 bp, synthetic construct
  misc_feature 1..23: note = Target sequence of sgRNA
  source 1..23: mol_type = other DNA
agccacaattacggtcttcccgg

SEQ ID NO: 8 - DNA, 23 bp, synthetic construct
  misc_feature 1..23: note = Target sequence of sgRNA
  source 1..23: mol_type = other DNA
cccctggctttcctggcactggg

SEQ ID NO: 9 - DNA, 23 bp, synthetic construct
  misc_feature 1..23: note = Target sequence of sgRNA
  source 1..23: mol_type = other DNA
ctggcagccacggcttcccctgg

SEQ ID NO: 10 - DNA, 23 bp, synthetic construct
  misc_feature 1..23: note = Target sequence of sgRNA
  source 1..23: mol_type = other DNA
tggcagccacggcttccccctgg

SEQ ID NO: 11 - DNA, 22 bp, synthetic construct
  misc_feature 1..22: note = Primer sequence
  source 1..22: mol_type = other DNA
aagccctcacgtctcaataacc

SEQ ID NO: 12 - DNA, 22 bp, synthetic construct
  misc_feature 1..22: note = Primer sequence
  source 1..22: mol_type = other DNA
gctttaagcagaccagtgggta